European Patent Application EP 4 574 981 A1, published June 25, 2025. Title: ANTI-FUNGAL VHH ANTIBODIES. Applicant: BIOTALYS NV. Application EP. The sequence listing filed with the application follows.

SEQUENCE LISTING (15 sequences)

SEQ ID NO: 1 - DNA, 384 bp, synthetic construct
  source 1..384: mol_type = other DNA
gacgtacagctgcaggagtctgggggaggattggtgcaggctgggggctctctgagactctcctgtgctgcctctagacgtaccggcactagatatgtgatggcctggttccgccaggctccagggaaggagcgtgagtttgtcgcaggtgttgactggagtggatcgggtcaatactatgcagagtccgtgaagggccgattcaccatctccaaagacaacaccaggaaaacggtgtatcttcagatgaacgccctgaaacctgaggacacggccgtttattactgtgcagcaacaaggcgactgtccgggcgtgcctacttgtgggccactgcttcgacgtatgactactggggccgggggacccaggtcaccgtctcctca

SEQ ID NO: 2 - protein, 128 aa, synthetic construct
DVQLQESGGGLVQAGGSLRLSCAASRRTGTRYVMAWFRQAPGKEREFVAGVDWSGSGQYYAESVKGRFTISKDNTRKTVYLQMNALKPEDTAVYYCAATRRLSGRAYLWATASTYDYWGRGTQVTVSS

SEQ ID NO: 3 - protein, 11 aa, synthetic construct
RRTGTRYVMAW

SEQ ID NO: 4 - protein, 19 aa, synthetic construct
AGVDWSGSGQYYAESVKGR

SEQ ID NO: 5 - protein, 19 aa, synthetic construct
TRRLSGRAYLWATASTYDY

SEQ ID NO: 6 - protein, 25 aa, synthetic construct
DVQLQESGGGLVQAGGSLRLSCAAS

SEQ ID NO: 7 - protein, 12 aa, synthetic construct
FRQAPGKEREFV

SEQ ID NO: 8 - protein, 31 aa, synthetic construct
FTISKDNTRKTVYLQMNALKPEDTAVYYCAA

SEQ ID NO: 9 - protein, 11 aa, synthetic construct
WGRGTQVTVSS

SEQ ID NO: 10 - DNA, 387 bp, synthetic construct
  source 1..387: mol_type = other DNA
gacgttcaactacaggagtctggtggcggtcttgttcaagctggaggatctcttaggctttcttgtgccgcatcccgtaggactggcactagatacgtgatggcatggtttaggcaagctcctggtaaagaaagggaatttgtcgctggagtagattggtccggctccggccaatactacgctgagtctgtgaagggtcgtttcactatctccaaggataatactaggaaaacggtatacttgcaaatgaacgctttgaaacctgaggatactgcagtttattactgcgctgcaaccaggaggctgtctggcagagcctatctgtgggctacagcatccacttacgactattggggaagaggtactcaagtgaccgtgtcctcataa

SEQ ID NO: 11 - DNA, 387 bp, synthetic construct
  source 1..387: mol_type = other DNA
gacgttcagttgcaagaatctggaggaggtttggttcaagctggtggttctttgagattgtcttgtgctgcttctagaagaactggtacaagatacgttatggcttggttcagacaagctccaggtaaagaaagagagtttgttgctggagtggattggagtggtagtggtcaatactacgctgaatctgttaagggtagatttactatttctaaagataacactagaaagactgtttaccttcaaatgaatgctttgaagcctgaggatactgccgtttactactgtgctgctactagaagattgtctggaagagcttatttgtgggctaccgcctctacttacgattattggggtagaggtactcaagttactgtctcttcttaa

SEQ ID NO: 12 - DNA, 387 bp, synthetic construct
  source 1..387: mol_type = other DNA
gacgttcaactccaagagtcaggtggtggtttggttcaggctggcggatctttaaggctttcttgtgcagcatccagacgtacaggaacaagatatgtgatggcctggttcagacaggctcctggtaaggaacgtgaattcgttgctggagtcgattggtcaggtagcggtcaatactacgcagaatccgttaagggtcgatttacgatcagtaaagataacactagaaaaaccgtctatttgcaaatgaatgctctgaaaccagaggacacagctgtatactactgcgcagctactagacgtttgagcggtagggcatacctatgggccactgcttcgacttatgactattggggtagaggaacacaagttaccgtgtcctcttaa

SEQ ID NO: 13 - DNA, 387 bp, synthetic construct
  source 1..387: mol_type = other DNA
gacgtccagctccaggagagcggcggcggcctcgtccaggctggcggcagcctccgcctcagctgcgccgcctctcgccgcaccggcacgcgctacgtcatggcctggttccgacaggcccctggcaaggagcgcgagttcgtcgccggcgtcgactggtccggcagcggccagtactacgccgagagcgtcaagggccgcttcaccatcagcaaggacaacacccgcaagaccgtctacctccagatgaacgccctcaagcctgaggacaccgccgtctactactgcgccgctacgcgccgactcagcggccgagcctacctctgggccaccgccagcacctacgactactggggccgaggcacccaggtcaccgtcagcagctaa

SEQ ID NO: 14 - DNA, 387 bp, synthetic construct
  source 1..387: mol_type = other DNA
gacgtccaattacaagagagtggcggcggattggtacaggctggaggatcactgagactatcgtgcgcagcaagccggcgaaccggtacccgatacgtgatggcgtggtttagacaggccccggggaaggaaagggaattcgttgccggcgttgactggtctggctccggccagtactatgccgagtctgtcaagggtcgcttcaccatctcgaaggataacacgcgcaagaccgtgtacctccaaatgaacgcccttaaacccgaggacactgctgtctactactgcgccgcgacgcgccgtctgagcggccgcgcgtatctctgggctacggcctccacttacgactattggggccgggggacacaggtcacagtcagctcctaa

SEQ ID NO: 15 - DNA, 387 bp, synthetic construct
  source 1..387: mol_type = other DNA
gatgtccaactgcaagaatcaggcggaggcctggttcaagcaggcggatcactgagactgtcatgcgcagcatcaagaagaacaggcacaagatatgttatggcgtggtttagacaagcaccgggaaaagaaagagaatttgttgcaggcgttgattggtcaggctcaggccaatattatgcagaatcagttaaaggacgcttcacgatcagcaaagataatacacgcaaaacagtctacctgcaaatgaatgcactgaaaccggaagatacagcagtctattattgcgcagcaacacgcagactgtcaggcagagcatatctgtgggcaacagcatcaacatatgattattggggcagaggcacacaagttacagtttcatcataa